European Patent Application EP 4 119 598 A1, published January 18, 2023. Title: COMPOSITE MATERIALS COMPRISING MECHANICAL LIGANDS. Applicant: Nanocore ApS. The sequence listing filed with the application follows.

SEQUENCE LISTING (51 sequences)

SEQ ID NO: 1 - protein, 7 aa, Artificial
  Synthetic peptide sequence
QLMHDYR

SEQ ID NO: 2 - protein, 9 aa, Artificial
  Synthetic peptide sequence
CPTSTGQAC

SEQ ID NO: 3 - protein, 9 aa, Artificial
  Synthetic peptide sequence
CTLHVSSYC

SEQ ID NO: 4 - protein, 12 aa, Artificial
  Synthetic peptide sequence
RLNPPSQMDPPF

SEQ ID NO: 5 - protein, 12 aa, Artificial
  Synthetic peptide sequence
QTWPPPLWFSTS

SEQ ID NO: 6 - protein, 12 aa, Artificial
  Synthetic peptide sequence
HTDWRLGTWHHS

SEQ ID NO: 7 - protein, 12 aa, Artificial
  Synthetic peptide sequence
ELWSIDTSAHRK

SEQ ID NO: 8 - protein, 11 aa, Artificial
  Synthetic peptide sequence
IFRLSWGTYFS

SEQ ID NO: 9 - protein, 12 aa, Artificial
  Synthetic peptide sequence
HWKHPWGAWDTL

SEQ ID NO: 10 - protein, 4 aa, Artificial
  Synthetic peptide sequence
ELWR

SEQ ID NO: 11 - protein, 7 aa, Artificial
  Synthetic peptide sequence
ELWRPTR

SEQ ID NO: 12 - protein, 7 aa, Artificial
  Synthetic peptide sequence
KPRSVSG

SEQ ID NO: 13 - protein, 9 aa, Artificial
  Synthetic peptide sequence
TGTGFGTCT

SEQ ID NO: 14 - protein, 9 aa, Artificial
  Synthetic peptide sequence
TGTGVGTCT

SEQ ID NO: 15 - protein, 9 aa, Artificial
  Synthetic peptide sequence
TGTGWGTCT

SEQ ID NO: 16 - protein, 9 aa, Artificial
  Synthetic peptide sequence
TGTGTGTCT

SEQ ID NO: 17 - protein, 9 aa, Artificial
  Synthetic peptide sequence
TGTGGGTCT

SEQ ID NO: 18 - protein, 9 aa, Artificial
  Synthetic peptide sequence
TGTGNGTCT

SEQ ID NO: 19 - protein, 9 aa, Artificial
  Synthetic peptide sequence
TGTGKGTCT

SEQ ID NO: 20 - protein, 9 aa, Artificial
  Synthetic peptide sequence
TGTGDGTCT

SEQ ID NO: 21 - protein, 14 aa, Artificial
  Synthetic peptide sequence
MHGKTQATSGTIQS

SEQ ID NO: 22 - protein, 42 aa, Artificial [sequence omitted]

SEQ ID NO: 23 - protein, 40 aa, Artificial
  Synthetic peptide sequence
DAEFRHDSGYEVHHQKLVFFAEDVGSNKGAIIGLMVGGVV

SEQ ID NO: 24 - protein, 9 aa, Artificial
  Synthetic peptide sequence
CHKKPSKSC

SEQ ID NO: 25 - protein, 12 aa, Artificial
  Synthetic peptide sequence
RKLPDAPGMHTW

SEQ ID NO: 26 - protein, 19 aa, Artificial
  Synthetic peptide sequence
SCSDCLKSVDFIPSSLASS

SEQ ID NO: 27 - protein, 7 aa, Artificial
  Synthetic peptide sequence
YLTMPTP

SEQ ID NO: 28 - protein, 7 aa, Artificial
  Synthetic peptide sequence
FSWEAFA

SEQ ID NO: 29 - protein, 7 aa, Artificial
  Synthetic peptide sequence
HLESTPG

SEQ ID NO: 30 - protein, 7 aa, Artificial
  Synthetic peptide sequence
GETRAPL

SEQ ID NO: 31 - protein, 7 aa, Artificial
  Synthetic peptide sequence
RHEPPLA

SEQ ID NO: 32 - protein, 7 aa, Artificial
  Synthetic peptide sequence
FPGRPSP

SEQ ID NO: 33 - protein, 7 aa, Artificial
  Synthetic peptide sequence
HKPDANR

SEQ ID NO: 34 - protein, 7 aa, Artificial
  Synthetic peptide sequence
FPGHSGP

SEQ ID NO: 35 - protein, 7 aa, Artificial
  Synthetic peptide sequence
THLPWQT

SEQ ID NO: 36 - protein, 7 aa, Artificial
  Synthetic peptide sequence
GETQCAA

SEQ ID NO: 37 - protein, 7 aa, Artificial
  Synthetic peptide sequence
HTAQSTA

SEQ ID NO: 38 - protein, 21 aa, Artificial
  Synthetic peptide sequence
VKTQATSREEPPRLPSKHRPG

SEQ ID NO: 39 - protein, 21 aa, Artificial
  Synthetic peptide sequence
PQAQDVELPQELQDQHREVEV

SEQ ID NO: 40 - protein, 105 aa, Artificial
  Synthetic peptide sequence
PQAQDVELPQELQDQHREVEVPQAQDVELPQELQDQHREVEVPQAQDVELPQELQDQHREVEVPQAQDVELPQELQDQHREVEVPQAQDVELPQELQDQHREVEV

SEQ ID NO: 41 - protein, 16 aa, Artificial
  Synthetic peptide sequence
SVSVGMKPSPRPGGGK

SEQ ID NO: 42 - protein, 12 aa, Artificial
  Synthetic peptide sequence
THRTSTLDYFVI

SEQ ID NO: 43 - protein, 21 aa, Artificial
  Synthetic peptide sequence
KTQATSESGSAGRQMFVADMG

SEQ ID NO: 44 - protein, 21 aa, Artificial
  Synthetic peptide sequence
KTQATSRGTRGMRTSGGFPVG

SEQ ID NO: 45 - protein, 21 aa, Artificial
  Synthetic peptide sequence
KTQATSVPRKAARRWEQVDSV

SEQ ID NO: 46 - protein, 21 aa, Artificial
  Synthetic peptide sequence
SKTSGRDQSKRVPRYWNVHRD

SEQ ID NO: 47 - protein, 20 aa, Artificial
  Synthetic peptide sequence
SKTSRESSAVQMGKARFLCT

SEQ ID NO: 48 - protein, 23 aa, Artificial
  Synthetic peptide sequence
CGSKGSIFRLSWGTYFSGSKGSC

SEQ ID NO: 49 - protein, 21 aa, Artificial
  Synthetic peptide sequence
SKTSRESSAVQMGKARFLCTH

SEQ ID NO: 50 - protein, 19 aa, Artificial
  Synthetic peptide sequence
CESSHWSAWWIRSNQSSSC

SEQ ID NO: 51 - protein, 12 aa, Artificial
  Synthetic peptide sequence
HWSAWWIRSNQS